European Patent Application EP 4 681 555 A2, published January 21, 2026. Title: Process for modifying gluco-oligosaccharides. Applicant: Cargill, Incorporated. The sequence listing filed with the application follows.

SEQUENCE LISTING (4 sequences)

SEQ ID NO: 1 - DNA, 2295 bp, Caldicellulosiruptor saccharolyticus
  source 1..2295: mol_type = other DNA
atgaaactgagcgaacgtgaatggctgattgaacaggataaactggaagcaagcggtaaatttgaaacctgttttgcactgaccaatggctatattggtattcgcggtattaacgaagaagtgttttgcgaagaaacaccgggtacatatattgccggtgtttttgataaaagcaccgcacaggttaccgaactggttaatctgccgaatccgattggtctgcgcatttatatcaatcgcgaatttctgaatccgctgaaatgcgaaatcctggaatttaaacgtgtgctggatctgaaacagggtattctgtatcgtaaactgcgtctgaaagatgtgaaaggtcgtattaccaccattgaaggttttcgttttgtgagcatgaacaacaaaaacctgatcgtgcagaaatatgatgtggtgtgtgaaaactatagcgcagttctgaatgtggaaagctttattgatgcaaccaccgtgaatagcaaagatgttccgaatgatcgcgtgaaacactatgagatcgataaaaagaaagatttcgccgatggtatctatctgggtattacgaccaaagacaaaaaatacaaagtgggtattgccagcagcaccaaagttctgctgaataatcagcgttgctattttaaccgcttcaccaaagatctgggctatatcattaccgaaaactttgaagttgaagccaaacagggtgaacgctatgaaattgaaaaactgaccgttctggttagcagccgtgaaaaaaatgttggtgatgtgtttgaaacgtgcaccaacaaactgaaagagttcgaaaccaaaagcgcagaaaaactgctgtttgaacacatcgaagaatataaacgtctgtgggatgttgcgaacattgatattgtgggtgatgaagttgccaacaaaagcgtgaaatttaacatcttccatctgattagcatggcgaatccggaagatgaacatgttagcctgggtgcaaaaggtctgcatggtgaaggttataaaggtcatgttttttgggataccgagatctttatgctgccgttctatatctataccaatccggcagcagcaaaagcaatgctgatgtatcgttataatctgctggatgccgcacgtgaaaatgcacgtaaaaacggctataaaggtgcacagtttccgtgggaaagtgcagataccggtgaagaagaaaccccgaaatggggttatgattatctgggcaatccggttcgtatttggaccggtgatatcgaatatcatatttcagccgatattgcctatgccgtgatgaattatgttcgtgcaaccgatgatattgacttcctgctgaattatggcagcgaaattatcattgaaaccgcacgtttttgggccagcatctgcaaatacaataaagaaaaaggccgttacgagatcaacgatgttattggtccggatgaatttcatgaacactgcaataataacgcctacaccaattatctggccaaatggaatctgctgaaagcaagcgaactgtgcaatctgctgctggaaaaatatccgaaatacttcgaaaagctgagcaaaaaaatcaacctgagtgatgaagaaccgtttgtgtggcaagaaattgcgagcaaaatctatattccgtatcacccggataaaaaactgatcgaacagttcgaaggctacttcaacctgaaagactttgtgatcaaagagtacgaccagaataatatgccggtttggcctgaaggtgtggaattagataaactgaataactaccagctgatcaaacaggccgatgttgttatgctgctgtatctgctgggtgaagaatttgatgatcagaccaaaaagatcaactacgattactatgagaaacgcaccatgcataaaagcagcctgagtccgagcatttatgcactgatgggtgttcgtgttggtgaaaccaatcgtgcctatattaactttatgcgtaccgcactgacagacctggaagataatcagggtaatacacatctgggcattcatgcagcaagcttaggtggcacctggcaggcactggtttttggttttggtggtattagcatcgaaaaagatgatgtgctgagcgttaatccgtggctgcctgaaaaatgggaaagtctgaaattttccatctggtggaaaggtaacctgctggatttcaaaatcacgaaagataacgtggaagtgaaaaagcgtgtggaaaaaggtaatgtgaaactgaaaatcaaaggccaagaagccatcattctcgagcaccaccaccaccaccactga

SEQ ID NO: 2 - protein, 764 aa, Caldicellulosiruptor saccharolyticus
MKLSEREWLIEQDKLEASGKFETCFALTNGYIGIRGINEEVFCEETPGTYIAGVFDKSTAQVTELVNLPNPIGLRIYINREFLNPLKCEILEFKRVLDLKQGILYRKLRLKDVKGRITTIEGFRFVSMNNKNLIVQKYDVVCENYSAVLNVESFIDATTVNSKDVPNDRVKHYEIDKKKDFADGIYLGITTKDKKYKVGIASSTKVLLNNQRCYFNRFTKDLGYIITENFEVEAKQGERYEIEKLTVLVSSREKNVGDVFETCTNKLKEFETKSAEKLLFEHIEEYKRLWDVANIDIVGDEVANKSVKFNIFHLISMANPEDEHVSLGAKGLHGEGYKGHVFWDTEIFMLPFYIYTNPAAAKAMLMYRYNLLDAARENARKNGYKGAQFPWESADTGEEETPKWGYDYLGNPVRIWTGDIEYHISADIAYAVMNYVRATDDIDFLLNYGSEIIIETARFWASICKYNKEKGRYEINDVIGPDEFHEHCNNNAYTNYLAKWNLLKASELCNLLLEKYPKYFEKLSKKINLSDEEPFVWQEIASKIYIPYHPDKKLIEQFEGYFNLKDFVIKEYDQNNMPVWPEGVELDKLNNYQLIKQADVVMLLYLLGEEFDDQTKKINYDYYEKRTMHKSSLSPSIYALMGVRVGETNRAYINFMRTALTDLEDNQGNTHLGIHAASLGGTWQALVFGFGGISIEKDDVLSVNPWLPEKWESLKFSIWWKGNLLDFKITKDNVEVKKRVEKGNVKLKIKGQEAIILEHHHHHH

SEQ ID NO: 3 - DNA, 2295 bp, Lactobacillus acidophilus
  source 1..2295: mol_type = other DNA
atgaaacgcatctttgaaatcgatccgtggaaagtgatcacccataaatttgatccgaaagacaaacgtctgcaagaaagcatgaccgcaattggcaatgattatatgggtatgcgtggcaattttgaagaaggttattcaggcgatagcctgcagggcacctatctggcaggcgtttggtttccggataaaaccgttgttggttggtggaaaaatggctatccgaaatactttggtaaaaccccgaatgcaccgagctttattggtattggcattaatgtgaatggcgagaaagttgatctggccaaagtgaaatttagcgattttgaactgagcctggatatgcatcagggtctgctgagccgtagctttatctatgaaggtaaagacgtgaaagtgaaactggaatttgaacgctttctgcatatcgttcagaaagaagcagcactgattaaagttaaagcaaccgttctggaaggccatgccaaaattgattttgatagcaccctggatggcaccgttgttaatgaagatagcaattatggtgatcgcttttggattccgctgggtgaagataaagatgaaaaaaccattcaggtgaaaaccaaaaagaacccgtatgatgttccgcagtttaccgttctgctgaaagaagccctgcgtaataacggtgttgcagttaatggtgaagttaccaccgaagatgcaaaactgagcgaacgttttagcgttgaactggatgaaggtcagagttatgaactggaaaaagatgttattgttgtgaccagccgtgatgtggaagaaaaagatcaggcagcagttgcaaataacctgatgagcaaactgcagaccaaaagctttgaagataatctggcagatcataccgaagcctggaaaaaacgttgggaaaccagtgatgttgaaatcagcggtgatgatgcagcacagcagggtattcgttttaacatttgtcagctgttcatgacctattacggcgaagataaacgcctgaatgttggtccgaaaggttttaccggtgaaaaatatggtggtgcaacctattgggataccgaggcatttattgttccgatgtatctggccgttaccaaaccgagcgttacccgtgcactgctgcagtatcgtcatgatcagttaccgggtgcatatcataatgcaaaagaacagggcctgcctggtgcactgtttccgatggttacctttaatggcattgagtgccataacgaatgggaaatcacctttgaagaaattcatcgtaatgccgatattccgcatgcaattgccatgtataccgattatacaggtgatgacagctacgtgaaaaatgaaggtatggatgttctggttggcaccgcacgtttttgggcagcacgtgttcattggagcaaaatgcgtaacaaatatgtgatgcatggtgttaccggtccgaacgaatatgaaaataatgtgaacaacaactggttcaccaataccatggcacgttggctgctgaaatataccctggaacgtctgccgctggcaaccaaagaagcacaagaacgcgtacgtgttaccgatgaagagaaagcaaaatggcaggatattgtggataatatgtatctgccggaagatgaagatctgggtatttttctgcagcaggatgatttcctggataaagatattcgtccggtgaccgaaattgaagatcagcgtccgattaatcagcattggagctgggataaaattctgcgtagcccgtttatcaaacaggcagatgttctgcagggtatctattttttcgatgatcagtatacgatggaccagaaagagaaaaacttcgatttttatgaaccgctgaccgtgcatgaaagcagcctgagtccgtgtatttatagcattatggcagcagaactgggcaaaaaagaaaaagcagttgaactgtatcagcgtaccgcacgtctggatctggataattacaataatgataccgtggatggcctgcatattaccagcatgagcggtagctggctggcaattgttcagggttttgcaggtatgcgttatgatcacgatcagctgaaatttaacccgtttgttccggatggttgggatcactatagcttcaaaataaactatcgtggtcgcctgattgaggtgtatgttgatcatgatgaatgcaaaattacactgctgagtggtgatgatctggaagttatggtgcatgataacaaactggatctgaaagagggtaaaaccaaatgtctgaaagccctcgagcaccaccaccaccaccactga

SEQ ID NO: 4 - protein, 764 aa, Lactobacillus acidophilus
MKRIFEIDPWKVITHKFDPKDKRLQESMTAIGNDYMGMRGNFEEGYSGDSLQGTYLAGVWFPDKTVVGWWKNGYPKYFGKTPNAPSFIGIGINVNGEKVDLAKVKFSDFELSLDMHQGLLSRSFIYEGKDVKVKLEFERFLHIVQKEAALIKVKATVLEGHAKIDFDSTLDGTVVNEDSNYGDRFWIPLGEDKDEKTIQVKTKKNPYDVPQFTVLLKEALRNNGVAVNGEVTTEDAKLSERFSVELDEGQSYELEKDVIVVTSRDVEEKDQAAVANNLMSKLQTKSFEDNLADHTEAWKKRWETSDVEISGDDAAQQGIRFNICQLFMTYYGEDKRLNVGPKGFTGEKYGGATYWDTEAFIVPMYLAVTKPSVTRALLQYRHDQLPGAYHNAKEQGLPGALFPMVTFNGIECHNEWEITFEEIHRNADIPHAIAMYTDYTGDDSYVKNEGMDVLVGTARFWAARVHWSKMRNKYVMHGVTGPNEYENNVNNNWFTNTMARWLLKYTLERLPLATKEAQERVRVTDEEKAKWQDIVDNMYLPEDEDLGIFLQQDDFLDKDIRPVTEIEDQRPINQHWSWDKILRSPFIKQADVLQGIYFFDDQYTMDQKEKNFDFYEPLTVHESSLSPCIYSIMAAELGKKEKAVELYQRTARLDLDNYNNDTVDGLHITSMSGSWLAIVQGFAGMRYDHDQLKFNPFVPDGWDHYSFKINYRGRLIEVYVDHDECKITLLSGDDLEVMVHDNKLDLKEGKTKCLKALEHHHHHH